European Patent Specification EP 3 986 138 B1, published January 28, 2026. Title: A BACILLUS STRAIN AND METHODS OF ITS USE FOR PLANT GROWTH PROMOTION. Applicant: Auburn University Bayer CropScience LP. The sequence listing filed with the application follows.

SEQUENCE LISTING (1 sequence)

SEQ ID NO: 1 - DNA, 1555 bp, Bacillus velezensis
tttatcggagagtttgatcctggctcaggacgaacgctggcggcgtgcctaatacatgcaagtcgagcggacagatgggagcttgctccctgatgttagcggcggacgggtgagtaacacgtgggtaacctgcctgtaagactgggataactccgggaaaccggggctaataccggatggttgtctgaaccgcatggttcagacataaaaggtggcttcggctaccacttacagatggacccgcggcgcattagctagttggtgaggtaacggctcaccaaggcgacgatgcgtagccgacctgagagggtgatcggccacactgggactgagacacggcccagactcctacgggaggcagcagtagggaatcttccgcaatggacgaaagtctgacggagcaacgccgcgtgagtgatgaaggttttcggatcgtaaagctctgttgttagggaagaacaagtgccgttcaaatagggcggcaccttgacggtacctaaccagaaagccacggctaactacgtgccagcagccgcggtaatacgtaggtggcaagcgttgtccggaattattgggcgtaaagggctcgcaggcggtttcttaagtctgatgtgaaagcccccggctcaaccggggagggtcattggaaactggggaacttgagtgcagaagaggagagtggaattccacgtgtagcggtgaaatgcgtagagatgtggaggaacaccagtggcgaaggcgactctctggtctgtaactgacgctgaggagcgaaagcgtggggagcgaacaggattagataccctggtagtccacgccgtaaacgatgagtgctaagtgttagggggtttccgccccttagtgctgcagctaacgcattaagcactccgcctggggagtacggtcgcaagactgaaactcaaaggaattgacgggggcccgcacaagcggtggagcatgtggtttaattcgaagcaacgcgaagaaccttaccaggtcttgacatcctctgacaatcctagagataggacgtccccttcgggggcagagtgacaggtggtgcatggttgtcgtcagctcgtgtcgtgagatgttgggttaagtcccgcaacgagcgcaacccttgatcttagttgccagcattcagttgggcactctaaggtgactgccggtgacaaaccggaggaaggtggggatgacgtcaaatcatcatgccccttatgacctgggctacacacgtgctacaatggacagaacaaagggcagcgaaaccgcgaggttaagccaatcccacaaatctgttctcagttcggatcgcagtctgcaactcgactgcgtgaagctggaatcgctagtaatcgcggatcagcatgccgcggtgaatacgttcccgggccttgtacacaccgcccgtcacaccacgagagtttgtaacacccgaagtcggtgaggtaaccttttaggagccagccgccgaaggtgggacagatgattggggtgaagtcgtaacaaggtagccgtatcggaaggtgcggctggatcacctcctttctaa